European Patent Application EP 4 610 359 A1, published September 3, 2025. Title: A microorganism for producing purine nucleotides and a method for producing purine nucleotides using the same. Applicant: CJ CheilJedang Corporation. The sequence listing filed with the application follows.

SEQUENCE LISTING (24 sequences)

SEQ ID NO: 1 - protein, 343 aa, Corynebacterium stationis
MHLQTSHKASRTHRGRRVALAALSIGALAFASACSTASSDEASDNGSEGSNGSDTLNIVTSTSIWGDIAQSVADSAEGADVEVTSIVEGNNMDPHHFEPTAADLARAAEADVIVVGGGGYDAWLYDTIEDQDKIIHALPLTAYSHDHGEESAEAEESHDHDHEHNHGEEGHSHEVSSIDGNEHIWYDPTAVMEVAHEIAEHINEANPDAQASDEEVVNKISDLDSRLHALPDVTYAQTEPIADYMLAHTDMTDATPEGYRHATLSHGEPAAADLAAFIDELKAGNVDVLIYNPQTQTDMTSRIRTTAEDEGIQIIEIGETPPDNQNFFEYFEEVVSNLESLEA

SEQ ID NO: 2 - DNA, 1032 bp, Corynebacterium stationis
  source 1..1032: mol_type = genomic DNA
atgcatttacagacttctcataaagcttcccgcactcaccgcggccgacgtgtagctttagctgcactaagcatcggcgcgctcgcctttgcatcggcatgctcaacggcatcttctgatgaagcatctgacaacggatcagaaggcagcaacggctctgacaccctgaacattgtcacttcgacatctatttggggcgatattgcacagtcggttgccgattcagcggaaggcgcggatgtagaagtcacctccattgttgaaggcaacaacatggacccgcaccacttcgaaccgaccgctgcggatttggcacgcgcggctgaagccgacgtgattgttgtgggcggcggcggatatgacgcctggctctacgacaccatcgaagaccaagacaagatcatccacgccctgccgctgaccgcgtacagccacgaccacggagaagaatctgcggaagcggaagaatcccatgatcacgaccatgagcataaccatggcgaggagggccactcgcatgaggtctcgtccatcgatggcaatgagcacatctggtacgacccaaccgcggtgatggaagtagcgcacgagattgctgagcacatcaacgaggccaacccagatgcgcaggcaagcgacgaagaagtagtcaacaagatctctgacttggattcacgcctgcacgcactgcctgatgttacttatgcacagaccgagccgattgcagactacatgctggcacacaccgacatgactgatgcaacgccagaaggctaccgccatgcaacgctcagccacggtgaaccagcagccgcagacttggcagcttttatcgatgagctcaaagcgggcaacgtggatgtgttgatctacaacccgcagacccaaaccgatatgacctcacggattcgcaccacggcggaagatgaaggcattcagattatcgagatcggtgagactcccccggataaccaaaacttctttgaatactttgaagaagtcgtatccaatctcgaatcgctcgaagcgtaa

SEQ ID NO: 3 - DNA, 38 bp, synthetic construct
  source 1..38: mol_type = other DNA
aattcgagctcggtaccctggcaaactcaaatccggct

SEQ ID NO: 4 - DNA, 35 bp, synthetic construct
  source 1..35: mol_type = other DNA
tttcttagcaggtatgcgtaggtcaaagtatcgcc

SEQ ID NO: 5 - DNA, 35 bp, synthetic construct
  source 1..35: mol_type = other DNA
tactttgacctacgcatacctgctaagaaatccac

SEQ ID NO: 6 - DNA, 35 bp, synthetic construct
  source 1..35: mol_type = other DNA
gattcggtctgcttgaaggatggttgggcttgcat

SEQ ID NO: 7 - DNA, 35 bp, synthetic construct
  source 1..35: mol_type = other DNA
agcccaaccatccttcaagcagaccgaatccatcg

SEQ ID NO: 8 - DNA, 38 bp, synthetic construct
  source 1..38: mol_type = other DNA
cgactctagaggatccccgtaccaagcgtgaagaggtt

SEQ ID NO: 9 - DNA, 38 bp, synthetic construct; identical to SEQ ID NO: 3
  source 1..38: mol_type = other DNA

SEQ ID NO: 10 - DNA, 35 bp, synthetic construct
  source 1..35: mol_type = other DNA
cgctgggatgtttctgcgtaggtcaaagtatcgcc

SEQ ID NO: 11 - DNA, 35 bp, synthetic construct
  source 1..35: mol_type = other DNA
tactttgacctacgcagaaacatcccagcgctact

SEQ ID NO: 12 - DNA, 35 bp, synthetic construct
  source 1..35: mol_type = other DNA
agtctgtaaatgcatgagtgtttcctttcgttggg

SEQ ID NO: 13 - DNA, 35 bp, synthetic construct
  source 1..35: mol_type = other DNA
cgaaaggaaacactcatgcatttacagacttctca

SEQ ID NO: 14 - DNA, 35 bp, synthetic construct; identical to SEQ ID NO: 6
  source 1..35: mol_type = other DNA

SEQ ID NO: 15 - DNA, 35 bp, synthetic construct; identical to SEQ ID NO: 7
  source 1..35: mol_type = other DNA

SEQ ID NO: 16 - DNA, 38 bp, synthetic construct; identical to SEQ ID NO: 8
  source 1..38: mol_type = other DNA

SEQ ID NO: 17 - DNA, 60 bp, synthetic construct
  source 1..60: mol_type = other DNA
acgacggccagtgaattcgagctcggtacccggggatcctgcgcggcaagaagggggacc

SEQ ID NO: 18 - DNA, 60 bp, synthetic construct
  source 1..60: mol_type = other DNA
tcactgaaagctttcacgtccatcgcactagtgcggccgcagtttgcaccggctttgcca

SEQ ID NO: 19 - DNA, 24 bp, synthetic construct
  source 1..24: mol_type = other DNA
actagtgcgatggacgtgaaagct

SEQ ID NO: 20 - DNA, 60 bp, synthetic construct
  source 1..60: mol_type = other DNA
gaccatgattacgccaagcttgcatgcctgcaggtcgactgctaatgcgccctgggaatg

SEQ ID NO: 21 - DNA, 40 bp, synthetic construct
  source 1..40: mol_type = other DNA
aaagccggtgcaaactgccatacctgctaagaaatccacc

SEQ ID NO: 22 - DNA, 39 bp, synthetic construct
  source 1..39: mol_type = other DNA
cgtccatcgcactagtgcaaggatggttgggcttgcatc

SEQ ID NO: 23 - DNA, 20 bp, synthetic construct
  source 1..20: mol_type = other DNA
gtctcgtccatcgatggcaa

SEQ ID NO: 24 - DNA, 20 bp, synthetic construct
  source 1..20: mol_type = other DNA
gctggcgacaactgtggtct